European Patent Specification EP 3 853 242 B1, published May 15, 2024. Title: HIGH THROUGHPUT METHOD AND SYSTEM FOR MAPPING INTRACELLULAR PHASE DIAGRAMS. Applicant: The Trustees Of Princeton University. The sequence listing filed with the application follows.

SEQUENCE LISTING (4 sequences)

SEQ ID NO: 1 - protein, 21 aa, Artificial Sequence
  sqTel
TTAGGGTTAGGGTTAGGGTTA

SEQ ID NO: 2 - protein, 18 aa, Artificial Sequence
  sqMaj
CAAGAAAACTGAAAATCA

SEQ ID NO: 3 - protein, 51 aa, Artificial Sequence
  Forward Primer
  misc_feature (25)..(25): Xaa can be any naturally occurring amino acid
CCCTTGGAGAACCACCTTGTTGGNXGTTTAAGAGCTATGCTGGAAACAGCA

SEQ ID NO: 4 - protein, 29 aa, Artificial Sequence
  Reverse Primer
GATCCTAGTACTCGAGAAAAAAAGCACCG